European Patent Specification EP 3 322 989 B1, published June 4, 2025. Title: NOVEL PEPTIDE COMBINATIONS FOR USE IN THE DIAGNOSIS OF SCHIZOPHRENIA. Applicant: Yeda Research and Development Co. Ltd. The sequence listing filed with the application follows.

SEQUENCE LISTING (30 sequences)

SEQ ID NO: 1 - protein, 5 aa, Artificial Sequence
  pentapeptide component
LLVVG

SEQ ID NO: 2 - protein, 5 aa, Artificial Sequence
  pentapeptide component
LLVGV

SEQ ID NO: 3 - protein, 5 aa, Artificial Sequence
  pentapeptide component
LLGVV

SEQ ID NO: 4 - protein, 5 aa, Artificial Sequence
  pentapeptide component
LVLVG

SEQ ID NO: 5 - protein, 5 aa, Artificial Sequence
  pentapeptide component
LVLGV

SEQ ID NO: 6 - protein, 5 aa, Artificial Sequence
  pentapeptide component
LGLVV

SEQ ID NO: 7 - protein, 5 aa, Artificial Sequence
  pentapeptide component
LVVLG

SEQ ID NO: 8 - protein, 5 aa, Artificial Sequence
  pentapeptide component
LVGLV

SEQ ID NO: 9 - protein, 5 aa, Artificial Sequence
  pentapeptide component
LGVLV

SEQ ID NO: 10 - protein, 5 aa, Artificial Sequence
  pentapeptide component
LVVGL

SEQ ID NO: 11 - protein, 5 aa, Artificial Sequence
  pentapeptide component
LVGVL

SEQ ID NO: 12 - protein, 5 aa, Artificial Sequence
  pentapeptide component
LGVVL

SEQ ID NO: 13 - protein, 5 aa, Artificial Sequence
  pentapeptide component
VLLVG

SEQ ID NO: 14 - protein, 5 aa, Artificial Sequence
  pentapeptide component
VLLGV

SEQ ID NO: 15 - protein, 5 aa, Artificial Sequence
  pentapeptide component
GLLVV

SEQ ID NO: 16 - protein, 5 aa, Artificial Sequence
  pentapeptide component
VLVLG

SEQ ID NO: 17 - protein, 5 aa, Artificial Sequence
  pentapeptide component
VLGLV

SEQ ID NO: 18 - protein, 5 aa, Artificial Sequence
  pentapeptide component
GLVLV

SEQ ID NO: 19 - protein, 5 aa, Artificial Sequence
  pentapeptide component
VLVGL

SEQ ID NO: 20 - protein, 5 aa, Artificial Sequence
  pentapeptide component
VLGVL

SEQ ID NO: 21 - protein, 5 aa, Artificial Sequence
  pentapeptide component
GLVVL

SEQ ID NO: 22 - protein, 5 aa, Artificial Sequence
  pentapeptide component
VVLLG

SEQ ID NO: 23 - protein, 5 aa, Artificial Sequence
  pentapeptide component
VGLLV

SEQ ID NO: 24 - protein, 5 aa, Artificial Sequence
  pentapeptide component
GVLLV

SEQ ID NO: 25 - protein, 5 aa, Artificial Sequence
  pentapeptide component
VVLGL

SEQ ID NO: 26 - protein, 5 aa, Artificial Sequence
  pentapeptide component
VGLVL

SEQ ID NO: 27 - protein, 5 aa, Artificial Sequence
  pentapeptide component
GVLVL

SEQ ID NO: 28 - protein, 5 aa, Artificial Sequence
  pentapeptide component
VVGLL

SEQ ID NO: 29 - protein, 5 aa, Artificial Sequence
  pentapeptide component
VGVLL

SEQ ID NO: 30 - protein, 5 aa, Artificial Sequence
  pentapeptide component
GVVLL